European Patent Application EP 4 147 576 A1, published March 15, 2023. Title: ENDOPHYTE COMPOSITIONS AND METHODS FOR IMPROVEMENT OF PLANT TRAITS. Applicant: Indigo Ag, Inc. The sequence listing filed with the application follows.

SEQUENCE LISTING (71 sequences)

SEQ ID NO: 1 - DNA, 20 bp, synthetic construct
  misc_feature 1..20: note = Synthetic Polynucleotide
  source 1..20: mol_type = other DNA
agagtttgatymtggctcag

SEQ ID NO: 2 - DNA, 19 bp, synthetic construct
  misc_feature 1..19: note = Synthetic Polynucleotide
  source 1..19: mol_type = other DNA
ggttaccttgttacgactt

SEQ ID NO: 3 - DNA, 19 bp, synthetic construct
  misc_feature 1..19: note = Synthetic Polynucleotide
  source 1..19: mol_type = other DNA
gtgycagcmgccgcggtaa

SEQ ID NO: 4 - DNA, 20 bp, synthetic construct
  misc_feature 1..20: note = Synthetic Polynucleotide
  misc_feature 8: note = n is a, c, g, or t
  source 1..20: mol_type = other DNA
ggactacnvgggtwtctaat

SEQ ID NO: 5 - DNA, 22 bp, synthetic construct
  misc_feature 1..22: note = Synthetic Polynucleotide
  source 1..22: mol_type = other DNA
cttggtcatttagaggaagtaa

SEQ ID NO: 6 - DNA, 20 bp, synthetic construct
  misc_feature 1..20: note = Synthetic Polynucleotide
  source 1..20: mol_type = other DNA
gctgcgttcttcatcgatgc

SEQ ID NO: 7 - DNA, 20 bp, synthetic construct
  misc_feature 1..20: note = Synthetic Polynucleotide
  source 1..20: mol_type = other DNA
gcatcgatgaagaacgcagc

SEQ ID NO: 8 - DNA, 17 bp, synthetic construct
  misc_feature 1..17: note = Synthetic Polynucleotide
  source 1..17: mol_type = other DNA
tcctgagggaaacttcg

SEQ ID NO: 9 - DNA, 20 bp, synthetic construct
  misc_feature 1..20: note = Synthetic Polynucleotide
  source 1..20: mol_type = other DNA
tgctggtagtgcgaatgaaa

SEQ ID NO: 10 - DNA, 19 bp, synthetic construct
  misc_feature 1..19: note = Synthetic Polynucleotide
  source 1..19: mol_type = other DNA
ctttcgggttccatcaggt

SEQ ID NO: 11 - DNA, 20 bp, synthetic construct
  misc_feature 1..20: note = Synthetic Polynucleotide
  source 1..20: mol_type = other DNA
ctaccgcaagagcaactgtg

SEQ ID NO: 12 - DNA, 20 bp, synthetic construct
  misc_feature 1..20: note = Synthetic Polynucleotide
  source 1..20: mol_type = other DNA
acttcctcctcctcctcctc

SEQ ID NO: 13 - DNA, 21 bp, synthetic construct
  misc_feature 1..21: note = Synthetic Polynucleotide
  source 1..21: mol_type = other DNA
gtcctcgcctaatcaggagtc

SEQ ID NO: 14 - DNA, 21 bp, synthetic construct
  misc_feature 1..21: note = Synthetic Polynucleotide
  source 1..21: mol_type = other DNA
tcctattccctgacgtgctac

SEQ ID NO: 15 - DNA, 20 bp, synthetic construct
  misc_feature 1..20: note = Synthetic Polynucleotide
  source 1..20: mol_type = other DNA
gaggaggaggaggagaggtt

SEQ ID NO: 16 - DNA, 20 bp, synthetic construct
  misc_feature 1..20: note = Synthetic Polynucleotide
  source 1..20: mol_type = other DNA
cgtccgtctcccagactatt

SEQ ID NO: 17 - DNA, 19 bp, synthetic construct
  misc_feature 1..19: note = Synthetic Polynucleotide
  source 1..19: mol_type = other DNA
atgtgcaaggccggtttcg

SEQ ID NO: 18 - DNA, 20 bp, synthetic construct
  misc_feature 1..20: note = Synthetic Polynucleotide
  source 1..20: mol_type = other DNA
tacgagtccttctggcccat

SEQ ID NO: 19 - DNA, 28 bp, synthetic construct
  misc_feature 1..28: note = Synthetic Polynucleotide
  source 1..28: mol_type = other DNA
tcgcgttcgttaacaaaatggaccgtat

SEQ ID NO: 20 - DNA, 28 bp, synthetic construct
  misc_feature 1..28: note = Synthetic Polynucleotide
  source 1..28: mol_type = other DNA
tcgccagacggcccagagccagacccat

SEQ ID NO: 21 - DNA, 20 bp, synthetic construct
  misc_feature 1..20: note = Synthetic Polynucleotide
  source 1..20: mol_type = other DNA
gartgyccdggdcayttygg

SEQ ID NO: 22 - DNA, 23 bp, synthetic construct
  misc_feature 1..23: note = Synthetic Polynucleotide
  misc_feature 3: note = n is a, c, g, or t
  misc_feature 9: note = n is a, c, g, or t
  source 1..23: mol_type = other DNA
ccngcdatntcrttrtccatrta

SEQ ID NO: 23 - DNA, 17 bp, synthetic construct
  misc_feature 1..17: note = Synthetic Polynucleotide
  source 1..17: mol_type = other DNA
acccgctgaacttaagc

SEQ ID NO: 24 - DNA, 17 bp, synthetic construct
  misc_feature 1..17: note = Synthetic Polynucleotide
  source 1..17: mol_type = other DNA
tcctgagggaaacttcg

SEQ ID NO: 25 - DNA, 23 bp, synthetic construct
  misc_feature 1..23: note = Synthetic Polynucleotide
  source 1..23: mol_type = other DNA
cccatrgcytgyttmcccatdgc

SEQ ID NO: 26 - DNA, 20 bp, synthetic construct
  misc_feature 1..20: note = Synthetic Polynucleotide
  source 1..20: mol_type = other DNA
gaygaymgwgatcayttygg

SEQ ID NO: 27 - DNA, 19 bp, synthetic construct
  misc_feature 1..19: note = Synthetic Polynucleotide
  source 1..19: mol_type = other DNA
gtagtcatatgcttgtctc

SEQ ID NO: 28 - DNA, 20 bp, synthetic construct
  misc_feature 1..20: note = Synthetic Polynucleotide
  source 1..20: mol_type = other DNA
cttccgtcaattcctttaag

SEQ ID NO: 29 - DNA, 21 bp, synthetic construct
  misc_feature 1..21: note = Synthetic Polynucleotide
  misc_feature 13: note = n is Queuosine
  source 1..21: mol_type = other DNA
tacctggttgatnctgccagt

SEQ ID NO: 30 - DNA, 23 bp, synthetic construct
  misc_feature 1..23: note = Synthetic Polynucleotide
  source 1..23: mol_type = other DNA
gtbcacctycaraccggycartg

SEQ ID NO: 31 - DNA, 26 bp, synthetic construct
  misc_feature 1..26: note = Synthetic Polynucleotide
  source 1..26: mol_type = other DNA
ccrgaytgrccraaracraagttgtc

SEQ ID NO: 32 - DNA, 17 bp, synthetic construct
  misc_feature 1..17: note = Synthetic Polynucleotide
  source 1..17: mol_type = other DNA
gtygayttcaaygtycc

SEQ ID NO: 33 - DNA, 20 bp, synthetic construct
  misc_feature 1..20: note = Synthetic Polynucleotide
  source 1..20: mol_type = other DNA
acaccdggdggrccgttcca

SEQ ID NO: 34 - DNA, 22 bp, synthetic construct
  misc_feature 1..22: note = Synthetic Polynucleotide
  source 1..22: mol_type = other DNA
cttccaggcatagtaatgtgga

SEQ ID NO: 35 - DNA, 23 bp, synthetic construct
  misc_feature 1..23: note = Synthetic Polynucleotide
  source 1..23: mol_type = other DNA
acttccactaccatgagcaattc

SEQ ID NO: 36 - DNA, 20 bp, synthetic construct
  misc_feature 1..20: note = Synthetic Polynucleotide
  source 1..20: mol_type = other DNA
ctcctcctcctcctcctgat

SEQ ID NO: 37 - DNA, 20 bp, synthetic construct
  misc_feature 1..20: note = Synthetic Polynucleotide
  source 1..20: mol_type = other DNA
tcacagagctacgcgacttg

SEQ ID NO: 38 - DNA, 1440 bp, Coniochaeta prunicola
  source 1..1440: mol_type = genomic DNA
tcttggtcatttagaggaagtaaaagtcgtaacaaggtctccgttggtgaaccagcggagggatcattacaagaagccgaaaggctacttcaaaccatcgtgaacttatccaagttgcttcggcggcgcggctcccctcgcggggtgccgcagccccgccccctcgggggtggtgggcgcccgccggaggtattaaactctcccgtattatagtggtatttctgagtaaaaacaaataagttaaaactttcaacaacggatctcttggttctggcatcgatgaagaacgcagcgaaatgcgataagtaatgtgaattgcagaattcagtgaatcatcgaatctttgaacgcacattgcgcccgctagtattctagcgggcatgcctgttcgagcgtcatttcaaccctcaagccctgcttggtgttggggccctacggctgccgtaggccctgaaaagaagtggcgggctcgctgcaactccgagcgtagtaattcattatctcgctagggaggcgcggcggtgctcctgccgttaaagaccatctttaaccaaaggttgacctcggatcaggtaggaatacccgctgaacttaagcatatcaataagcggaggaaaagaaaccaacagggattgccctagtaacggcgagtgaagcggcaacagctcaaatttgaaatctggcttcggcccgagttgtaatttgtagaggatgcttttggtgaggtgccttctgagttccctggaacgggacgccagagagggtgagagccccgtatagtcggccaccgatcctctgtaaagctccttcgacgagtcgagtagtttgggaatgctgctcaaaatgggaggtatatctcttctaaagctaaatataggccagagaccgatagcgcacaagtagagtgatcgaaagatgaaaagcactttgaaaagagggttaaatagcacgtgaaattgttgaaagggaagcgcttgtgaccagacttgcgccgggctgatcatccagtgttctcactggtgcactcgacccggctcaggccagcgtcggttctcgcagggggataaaagcttcgggaacgtggcaccttcgggtgtgttatagcccgctgcttaataccccggtggggaccgaggttcgcgctctgcaaggacgctggcataatggtcatcagcgacccgtcttgaaacacggaccaaggagtcgaggttttgcgcgagtgtttgggtgtaaaacccgcacgcgtaatgaaagtgaacgtaggtgagagcttcggcgcatcatcgaccgatcctgatgtattcggatggatttgagtaagagcgtatagcctcggacccgaaagatggtgaactatgcctgaatagggggaagccagaggaaactctggtggaggctcgcagcggttctgacgtgcaaatcgatcgtcaaatttgggca

SEQ ID NO: 39 - DNA, 922 bp, Coniochaeta prunicola
  source 1..922: mol_type = genomic DNA
tcctgagggaaacttcggcggtaaccagctactagatggttcgattagtctttcgcccccatgcccaaatttgacgatcgatttgcacgtcagaaccgctgcgagcctccaccagagtttcctctggcttcaccctattcaggcatagttcaccatctttcgggtccgaggctatacgctcttactcaaatccatccgaatacatcaggatcggtcgatgatgcgccgaagctctcacctacgttcactttcattacgcgtgcgggttttacacccaaacactcgcgcaaaacctcgactccttggtccgtgtttcaagacgggtcgctgatgaccattatgccagcgtccttgcagagcgcgaacctcggtccccacaggggtattaagcagcgggctataacacacccgaaggtgccacgttcccgaagcttttatccccctgcgagaaccgacgctggcctgagccgggtcgagtgcaccagtgagaacactggatgatcagcccggcgcaagtctggtcacaagcgcttccctttcaacaatttcacgtgctatttaaccctcttttcaaagtgcttttcatctttcgatcactctacttgtgcgctatcggtctctggcctatatttagctttagaagagatatacctcccattttgagcagcattcccaaactactcgactcgtcgaaggagctttacagaggatcggtggccgactatacggggctctcaccctctctggcgtcccgttccagggaactcagaaggcacctcaccaaaagcatcctctacaaattacaactcgggccgaagccagatttcaaatttgagctgttgccgcttcactcgccgttactagggcaatccctgttggtttcttttcctccgcttattgatatgcttaagttcagcgggta

SEQ ID NO: 40 - DNA, 1151 bp, Coniochaeta prunicola
  source 1..1151: mol_type = genomic DNA
cttccgtcaatttctttaagtttcagccttgcgaccatactccccccagaacccagaaactttactttcgtgtaaggtgccgaacgagtcaaaatataacatcgtccgatccctagtcggcatagtttatggttaagactacgacggtatctgatcgtcttcgatcccctaactttcgttcctgattaatgaaaacatccttggcaaatgctttcgcagtagttagtcttcaataaatccaagaatttcacctctgacaattgaatactgatgcccccgactgtccctattaatcattacggcggtcctagaaaccaacaaaatagaaccacacgtcctattctattattccatgctaatgtattcgagcataggccttctttaagcgatctaatttgttcaaagtaaaagtcctggttccccgacacacccagtgaagggcatgcggttccccagagggaaaggcccggccggaccagtgcacgcggtgaggcggaccggccagccaggcccaaggttcaactacgagctttttaactgcaacaactttaatatacgctattggagctggaattaccgcggctgctggcaccagacttgccctccaattgttcctcgttaagggatttaaattgtactcattccaattacaagacccaaaagagccctgtatcagtatttattgtcactacctccccgaatcgggattgggtaatttgcgcgcctgctgccttccttggatgtagtagccgtttctcaggctccttctccggggtcgagccctaaccctccgttacccgttgtcaccatggctggccaagacccagccgtcgaaagttgatagggcagaaatttgaatgaaccatcgccggcgcaaggccgtgcgattcgagaagttattatgaatcaccagagagccccgaagggcattggtttttaatctaataaatacatcccttccgaagtcgggatttttagcatgtattagctctagaattaccacggttatccaagtagtaaggtactatcaaataaacgataactgatttaatgagccattcgcagtttcgcggtataattgcttatacttagacatgcatggcttaatctttgagacaagcatatgactactggcagaatcaaccaggtaa

SEQ ID NO: 41 - DNA, 604 bp, Coniochaeta prunicola
  source 1..604: mol_type = genomic DNA
tgctggtagtgcgaatgaaaatggctggttccaggatataacgggtaatcgactgcactttaacaaggctatgcgagtactttgcgaccatggtcttgcagaagcagatccgccgacgaaagagcacggttcggagtctggagggtacagtgtgcacggatgtgtgcactcctggatggtaaacgtcctcaaccagacaggagatgcggagatggcacgtctggctttgaggtgtgtggctagccatgtgccaagcacggaggagggtgagtattggcgggtacagcggcgcctccttctgcacgcagaccaatgcttgaaattgatggaagagggtcaggaggaggaaggcaatggatgggtattccataatctaggagatctctacaaagcccaagggcggttcaaggaagcagaagccatgtacgagcgggcgcttcgaggcaaggagaaggcatggggaccagaccacacgtcgacactcgacacagtcaacaatctgggtctcgtcgccgacaacaaagccagccacaccaaacatcaagttccattctcgttccccgtctttgtcgtgtggcagacaaaacctgatggaacccgaaag

SEQ ID NO: 42 - DNA, 1428 bp, Curvularia spicifera
  source 1..1428: mol_type = genomic DNA
aggtgaacctgcggagggatcattacacaataaaatacgaaggccgttcgcggctggactatttattacccttgtcttttgcgcacttgttgtttcctgggcgggttcgctcgccaccaggaccacaatataaaccttttttatgcagttgcaatcagcgtcagtataacaaatgtaaatcatttacaactttcaacaacggatctcttggttctggcatcgatgaagaacgcagcgaaatgcgatacgtagtgtgaattgcagaattcagtgaatcatcgaatctttgaacgcacattgcgccctttggtattccaaagggcatgcctgttcgagcgtcatttgtaccctcaagctttgcttggtgttgggcgtttttgtctttggcccgccaaagactcgccttaaaatgattggcagccggcctactggtttcgcagcgcagcacatttttgcgcttgcaatcagcaaaagaggacggcaatccatcaagactccttctcacgtttgacctcggatcaggtagggatacccgctgaacttaagcatatcaataagcggaggaaaagaaaccaacagggattgccctagtaacggcgagtgaagcggcaacagctcaaatttgaaatctggctctttcagagtccgagttgtaatttgcagagggcgctttggctttggcagcggtccaagttccttggaacaggacgtcacagagggtgagaatcccgtacgtggtcgctagctattgccgtgtaaagccccttcgacgagtcgagttgtttgggaatgcagctctaaatgggaggtaaatttcttctaaagctaaatattggccagagaccgatagcgcacaagtagagtgatcgaaagatgaaaagcactttggaaagagagtcaaacagcacgtgaaattgttgaaagggaagcgcttgcagccagacttgcttgcagttgctcatccgggcttttgcccggtgcactcttctgcaggcaggccagcatcagtttgggcggtgggataaaggtctctgtcacgtaccttccttcgggttggccttataggggagacgccataccaccagcctggactgaggtccgcgcatctgctaggatgctggcgtaatggctgtaagcggcccgtcttgaaacacggaccaaggagtctaacatctatgcgagtgtttgggtgtcaagcccgagcgcgtaatgaaagtgaacggaggtgggaacccgcaagggtgcaccatcgaccgatcctgaagtttacggaaggatttgagtaagagcatggctgttgggacccgaaagatggtgaactatgcttgaatagggtgaagccagaggaaactctggtggaggctcgcagcggttctgacgtgcaaatcgatcgtcaaatttgggcataggggcgaaagactaatcgaa

SEQ ID NO: 43 - DNA, 1197 bp, Curvularia spicifera
  source 1..1197: mol_type = genomic DNA
cccatagcttgcttacccatagcagattggtatgtgttacggggcgactggttgtgatctgggaagggaatgatactggcgcaaatacccaagatcatagctgggtgaatctcacaatgggtgtaggcgtggatgcgaggatccggtagtggcttgagacggcggagtcgatccttgccttcagtagatcgctcagctgcaggcaagcccatcttcatttctcgccattcttccaagtcctcgggagagaatgttatcattgcagtttcttcttcctcggcatcgaggtattcaacgacaccgtcttgaatgagacctctccagccgtatgtagcctgctcgacttcctcttgactccagccttgtcttgtactggtctcttgctgttcagccttgagcttgttgctgatttccttggtaaagatgaggtggttccggtttggctttcgaatatcgttttctacaacgaacaaaggcctcatgacacgacccgcatctgtgaatatcttgaactctctgtcgcgaatatcacgaatcaaactcatctcgtaagacagagtaccattgcggcgaagctcctgcacgactgtgacaagctgctgagcatttgaatgaacaccaacccagacaccgttaacgaagaccttggtcgcatccgggttctggttctggtcgtactcctcgagaagttgcatgttacgttgtgtcatgaagtcgataatgggcgatgcatcgctaccaacactgacataacacataagagacaagttcttgaccagaccgcaagcctgtccttcgggcgtctcagcagggcagacaagaccccaatgagagttgtgaagctgtcgcggctttgccaacttaccatcacgtccaacgggggtgttcgttcgacgcagatgggatagtgtggaggcataggtgtatcggttcaacacctgcgaaacaccagccttggcagatgcagccttcttctgatcaccccaattgcctgtagccagagagtacttcaggccgtttgtgatgatgctggctttcacagccatttgaacattgaagtcttggttgttttccacgcaccgctggaggtacttgtagacatccttggtgagcttcaggaacaagattcggaacaagttggcaatcagaggtccagccagatctagtcgcttctttccaaagtgatcacgatcgtcc

SEQ ID NO: 44 - DNA, 387 bp, Curvularia spicifera
  source 1..387: mol_type = genomic DNA
gttcacctccagaccggtcaatgcgtaagtctcgcgccgcctgaaaacaccacgggaacgactgctaacagccgctacagggtaaccaaattggtgccgccttctggcagaccatttccggcgagcatggcctcgacggctctggtgtctacaacggcacctctgaccttcagctcgagcgcatgaacgtctacttcaacgaagtacgtccctcggtgaagctccaacagacaaaagaccaatactgatgtgcagcaggcttccaacaacaagttcgtgccccgtgccgtcctcgtcgatctcgagcctggtactatggacgctgtccgcgctggtccctttggtcagctcttccgccccgacaacttcgtcttcggccagtcgggt

SEQ ID NO: 45 - DNA, 590 bp, Curvularia spicifera
  source 1..590: mol_type = genomic DNA
ctaccgcaagagcaactgtgcaagtccagcttcagtccctttcgatccccctcgcccaggaagagattcacccacgagcgcaaccagtccgaggcggtccagcgtccacgtcctatgagcgtttgcagcaactcgccagcagttcagcacaccaaaagagcctccatctacgtctccgacgcttccatcatcctagcgcaacgctcacccatggcttctccggtttccccaccagactccatgtcctcccccatccatgaatcgtctgatgccgtcgaccactatgctatcctggagatcacccctagagcaactaccgatgaggtcaaggctgcctaccgccgactacgggtcgtctacttctcaagtgacgcgaagaagtaccgagcactgcaggcggccttcgacgtcttgatggacccgcaatcccgcgaagcttacgacgcaacctatcaaccaactgccgcagcaccagtatcgctcgctagcattggtgagatcctggactcggggaagctatggcgacaggacagcgcccacggagacgacccagtaatcccagaagaggaagaggaggaggaggaggaagt

SEQ ID NO: 46 - DNA, 1458 bp, Acremonium alternatum
  source 1..1458: mol_type = genomic DNA
tcttggtcatttagaggaagtaaaagtcgtaacaaggtctccgttggtgaaccagcggagggatcattaccgagtgtaaaaactcccaaaccattgtgaacttaccactgttgcttcggcggcctcgccccgggcgcgttcgcgcggcccggacccaggcgtccgccggaggctccaaactcttgtcttttagtgtatttctgagtggcataagcaaataaatcaaaactttcagcaacggatctcttggttctggcatcgatgaagaacgcagcaaaatgcgataagtaatgtgaattgcagaattcagtgaatcatcgaatctttgaacgcacattgcgcccgccagtattctggcgggcatgcctgtctgagcgtcatttcaaccctcaggacccgttcgcgggacctggcgttggggatcagcctgcccctggcggcggctggccctgaaatccagtggcggttccctcgcgaactcctccgtgcagtaattaaacctctcgcggcaggatagcggttgaaccacgccgttaaaccccccacttctcaaggttgacctcagatcaggtaggaatacccgctgaacttaagcatatcaataagcggaggaaaagaaaccaacagggattgccctagtaacggcgagtgaagcggcaacagctcaaatttgaaatctggcctcacggtccgaattgtaatttgtagaggatgtttctggcgacgtgtcttccgagttccctggaacgggacgccatagagggtgagagccccgtccggtcgtacacctagcctctgtgaaactccttcgacgagtcgagtagtttgggaatgctgctctaaatgggaggtatacgtcttctaaagctaaataccggccagagaccgatagcgcacaagtagagtgatcgaaagatgaaaagcactttgaaaagagggttaaatagtacgtgaaattgctgaaagggaagcgcttatgaccagacttgggctcggtgaatcatccggcgttctcgccggtgcactttgccgtcccaggccagcatcagttcgcgccgggggataaaggtttcgggaatgtagctccttcgggagtgttatagcccgttgcgtaataccctggcgtggactgaggtccgcgctctgcaaggatgctggcgtaatggtcatcagtgacccgtcttgaaacacggaccaaggagtcgtcttcgtatgcgagtgttcgggtgtcaaacccctacgcgtaatgaaagtgaacgtaggagagagcttcggcgcatctccgaccgatcctgatgttctcggatggatttgagtaagagcatacggggccggacccgaaagaaggtgaactatgcctgtatagggtgaagccagaggaaactctggtggaggctcgcagcggttctgacgtgcaaatcgatcgtcaaatatgggcatgggggcgaaagactaatc

SEQ ID NO: 47 - DNA, 290 bp, Acremonium alternatum
  source 1..290: mol_type = genomic DNA
atgtgcaaggccggtttcgccggtgacgatgctccccgagctgttttccgtaagtcaaccccactttcgcttcccaagctcctaatcgcccacacctggcgatatgggctttgggggcctgtaagcagccgacacaagactaacgcgatgcgccagcttccattgtcggtcgcccccgtcaccatgggtaagtacgcgcgcaaatgacacctgtcagccccctcgacgagcggcacaggctctgaccattcgatagtatcatgattggtatgggacagaaggactcgtac

SEQ ID NO: 48 - DNA, 380 bp, Acremonium alternatum
  source 1..380: mol_type = genomic DNA
ccggactggccgaagacgaagttgtcgggacggaagagctgaccgaaaggaccggcgcggacggcatccatggtaccgggctcgagatcgacgaggacagcgcgaggaacgtacttgttgccagaggcctacagagggtcagcttggccacagactgcgggatactccaaattgctcacctcgttgaagtagacgctcatgcgctcgagctggagctcagaggtgccgttgtagacaccgttgctgtcgaggccatgctcgccagagatggtctgccagaaggcagcaccaatctggttaccctgctcggaggttagacatggtaggcgatatcacatatggcggaagtacttacgcactgaccggtctggaggtgaacc

SEQ ID NO: 49 - DNA, 1231 bp, Acremonium alternatum
  source 1..1231: mol_type = genomic DNA
gatgatcgtgatcacttcgggaaaaagcgccttgacctggctgggcccctcttagctaaattgttccgcaacattattcgcaggatcaacaacgagctgtcgacctacctcaggcgatgtgtcgagggcggcaggaacttcaacctcgctgtcggcatcaagcctggcacactgtcgaacgggttgaagtactctttggcaacaggcaactggggagaccaaaagaaggcaatgagctcggttgctggagtgtcccaggttctcaaccgctacacatttgcgtcaaccttgtctcatttgaggcgcaccaacacccccattggccgtgatggaaagctggcgaagcctcggcagctacacaacacgcattggggtcttgtgtgtcccgccgagacccccgagggtcaggcttgtggtttggtgaagaacctgtcactgatgtgtcacgtttccgttggcacacctagcgaacctctctacggatacttcatcaaccgtggcatggaagtgctcgaagagtacgagccccagcggttccccaacgccaccaaggtgttcatcaacggtgcctgggtcggtgtgcacacaagcccgaaagatctcgtggatagcatcatgcatctgcggcgctatggtgacctgaaccatgaagcttccgtcatccgcgacattcgggatcgagagttcagggtcgtcacggatgctggtcgtgttatgcgcccagtattcaccgtgcagcaagaagacaagctagacgggcccgagaagggctcgttgtgcatgaccaaggagcatcttgccggtttggatgactggcatctggtcaacgaggagagggaagagatggccacgggctgggagtacctcgtgaagagtgggtgtattgagtacttggacgccgaagaagaagagacggcaatgatttgcatgacaccagaagacttggagtcttaccgcaaggagaagtacctcgatcagaaaccccaggagcacaacgtggaagccgagcccaacaagcgactcaagacgaagaccaacccgacgacacacatgtacacccactgcgagattcatcccagtatgatcctcggtatctgcgccagcatcatccccttcccggatcataaccaggcatgtctctacgccaccagacctcgagattacttactaatattgcatctagtcgccccgtaatacttaccaatctgccatgggcaagcaggccatgggc

SEQ ID NO: 50 - DNA, 790 bp, Acremonium alternatum
  source 1..790: mol_type = genomic DNA
gaatgccccggtcattttggtcacatcgagctggcaaagcccgtttaccaccccggcttcatcaagaaagtcaagaagattttggagattgtctgccacaactgcagcaaggtcttggccgatgaagttggtctcacctgatccatgtcttgttccttagatgctaacatggacctctcagagcgaccccgagtttgtcactgcgatccgtacgcgcgacccgaaagtccgcttccagcgagtctgggctgtgtgcaagaagaagcggaagtgtgagaacgaggatcgccaagacaagaaggaagaggagttcgcgcccggcatgaagccgcagacgcacaaccacggcggctgtggaaacgagatgcccgcggttcgtcaagctggtttgcgtctcaacgcgcagttcgagatcaaggaagagggcggagctaagcgcaaggatactcaagttatcctgcccgaccaagctcacacaatcctgcggcggatatcggaacaggacctccgacacatgggcctcaactcagagtatgcccgcccagagtggatggttcttaccgtccttccggtccccccgcctcccgttcgtccaagtatttccatggacggcactggcacgggaatgcggaacgaggatgatttgacttacaagcttggtgatatcatccgagccaacggaaacgtcaagcaggctatccgcgaaggctcgccggcccacattgctcgcgatttcgaagagctgctccagtaccatgtagccacctacatggataatgatattgctgga

SEQ ID NO: 51 - DNA, 593 bp, Acremonium alternatum
  source 1..593: mol_type = genomic DNA
gtcctcgcctaatcaggagtcactagacgacatacccgaggacgacatgatgggcgaccttgcgcttggcctttcgagcagcttcaagcaacacgccctccggaactcaaagggcaagaccttctgggataccttctccgagacgagcagtgtcgcaggaccgagaaccacgccacctccgccgggagtgatggctcgacgtccatcgtccggcaggagtgaggatgtgaccatggattcgccgctccagcaaagcagcatgccttggctacaaacacggcacctttccgactcccagcgctcggactcggcacctgcggccaaggagaaggactccccggcccagccacccaccgctgcagagataacgcgccgaatcaacaacaaacgccgccgtgacgatgacttcgacccggtgagcttcaaacgccgcgcagtgagtcccgggctcagcgtccacaactcgccgctcccgcagagcccaatgcagcagagcggtgcgccatggggttccaggccgggaagcaatgggggcgacaaggcgggaagcagtgcacctagcgaatctggtggtagcacgtcagggaatagga

SEQ ID NO: 52 - DNA, 1453 bp, Chaetomium globosum
  source 1..1453: mol_type = genomic DNA
tcttggtcatttagaggaagtaaaagtcgtaacaaggtctccgttggtgaaccagcggagggatcattacagagttgcaaaactccctaaaccattgtgaacgttacctataccgttgcttcggcgggcggccccggggtttaccccccgggcgcccctgggccccaccgcgggcgcccgccggaggtcaccaaactcttgataatttatggcctctctgagtcttctgtactgaataagtcaaaactttcaacaacggatctcttggttctggcatcgatgaagaacgcagcgaaatgcgataagtaatgtgaattgcagaattcagtgaatcatcgaatctttgaacgcacattgcgcccgccagcattctggcgggcatgcctgttcgagcgtcatttcaaccatcaagcccccgggcttgtgttggggacctgcggctgccgcaggccctgaaaagcagtggcgggctcgctgtcgcaccgagcgtagtagcatacatctcgctctggtcgcgccgcgggttccggccgttaaaccaccttttaacccaaggttgacctcggatcaggtaggaagacccgctgaacttaagcatatcaataagcggaggaaaagaaaccaacagggattgccctagtaacggcgagtgaagcggcaacagctcaaatttgaaatctggcttcggcccgagttgtaatttgcagaggaagctttaggcgcggcaccttctgagtcccctggaacggggcgccatagagggtgagagccccgtatagttggatgcctagcctgtgtaaagctccttcgacgagtcgagtagtttgggaatgctgctcaaaatgggaggtaaatttcttctaaagctaaataccggccagagaccgatagcgcacaagtagagtgatcgaaagatgaaaagcactttgaaaagagggttaaatagcacgtgaaattgttgaaagggaagcgcttgtgaccagacttgcgccgggcggatcatccggtgttctcaccggtgcactccgcccggctcaggccagcatcggttctcgcggggggataaaggtcctgggaacgtagctcctccgggagtgttatagcccggggcgtaatgccctcgcggggaccgaggttcgcgcatctgcaaggatgctggcgtaatggtcatcagcgacccgtcttgaaacacggaccaaggagtcaaggttttgcgcgagtgtttgggtgtaaaacccgcacgcgtaatgaaagtgaacgtaggtgagagcttcggcgcatcatcgaccgatcctgatgttttcggatggatttgagtaggagcgttaagccttggacccgaaagatggtgaactatgcttggatagggtgaagccagaggaaactctggtggaggctcgcagcggttctgacgtgcaaatcgatcgtcaaatctgagcatgggggcgaaaga

SEQ ID NO: 53 - DNA, 266 bp, Chaetomium globosum
  source 1..266: mol_type = genomic DNA
atgtgcaaggccggtttcgccggtgatgatgcaccccgcgctgttttccgtaagtctcccagccccggccccggcccggtcggcgataagccgagctccggacgctcgttggcacaaacagacaagctaacagcgccgtttagcgtcgattgtcggtcgtccccgtcaccatgggtaggctttcagttccggtatctctgcgatatggggtcgctggctaacgcgccgctagtattatgatcggtatggggcagaaggactcgtac

SEQ ID NO: 54 - DNA, 923 bp, Chaetomium globosum
  source 1..923: mol_type = genomic DNA
tcctgagggaaacttcggcggtaaccagctactagatggttcgattagtctttcgcccccatgctcagatttgacgatcgatttgcacgtcagaaccgctgcgagcctccaccagagtttcctctggcttcaccctatccaagcatagttcaccatctttcgggtccaaggcttaacgctcctactcaaatccatccgaaaacatcaggatcggtcgatgatgcgccgaagctctcacctacgttcactttcattacgcgtgcgggttttacacccaaacactcgcgcaaaaccttgactccttggtccgtgtttcaagacgggtcgctgatgaccattacgccagcatccttgcagatgcgcgaacctcggtccccgcgagggcattacgccccgggctataacactcccggaggagctacgttcccaggacctttatccccccgcgagaaccgatgctggcctgagccgggcggagtgcaccggtgagaacaccggatgatccgcccggcgcaagtctggtcacaagcgcttccctttcaacaatttcacgtgctatttaaccctcttttcaaagtgcttttcatctttcgatcactctacttgtgcgctatcggtctctggccggtatttagctttagaagaaatttacctcccattttgagcagcattcccaaactactcgactcgtcgaaggagctttacacaggctaggcatccaactatacggggctctcaccctctatggcgccccgttccaggggactcagaaggtgccgcgcctaaagcttcctctgcaaattacaactcgggccgaagccagatttcaaatttgagctgttgccgcttcactcgccgttactagggcaatccctgttggtttcttttcctccgcttattgatatgcttaagttcagcgggtc

SEQ ID NO: 55 - DNA, 797 bp, Chaetomium globosum
  source 1..797: mol_type = genomic DNA
gagtgtccaggtcactttggccacattgagctatccagacccgttttccaccccgggttcatcaggcgtgtcaaaaagttgctcgagatggtctgccacaactgcagcaaggtgttggctgatcgtgttagtgcaccttgcctgaccgagtgatgatttgttttggcatgctaactcttcaccaggaggacgagcaatatgctgctgccatgcggattcgggaccccaaagtacgcttcaagcgagtttgggatatttgcaagagtaagaagcgctgcgaaaacgaagtgcgcaaggggaaagatggcgagttcaaacccgacagcgaaaaccaagccgcagagggtggccatggaggatgtggcaacacgcagccagtcattcgccagcaggctctcaccctgtggggcagcgtcgagaccaaggacgaggatggtgtgaagaccaaggagaagaaggtcatcaccccagaaatggccctgaacatcttccgtcgcatgtcggacgacgagatgattgacattggcctcaatatttcccaagctcgtccggaatggatgatcatcacggttcttcctgtcccgcctcctccggtgcgccccagtatttccatggacggaactggaacaggcttgcggaatgaggacgatctgacgtataaactcggcgatatcatccgcgccaatggcaacgtccgccaggctattgccgagggctctcctcagcatatcatcaccgactttgagaacctactccagtaccacgtcgctacgtacatggataatgacatcgccggt

SEQ ID NO: 56 - DNA, 1132 bp, Chaetomium globosum
  source 1..1132: mol_type = genomic DNA
cttccgtcaatttctttaagtttcagccttgcgaccatactcccccaggagcccaaacattttgatttatcgtaaggtgccgaacgggtcaaaaaataacgccgtccgatccctaatcggcatagtttaggttaagactacgacggtatctgatcgtattcgatcccctaactttcgttcctgattaatgaaaacatccttggcaaatgctttcgcagtagttagtcttcaataaatccaagaatttcacctctgacaattgaatactgatgcccccgactgtccctattaatcattacggcggtcctagaaaccaacaaaatagaaccacacgtcctattctattattccatgctaatgtattcgagcataggccttctttaagcgatctaatttgttcagagtaaaagtcctggttccccggcacacccagtgaagggcatgcggttctccagaaggaaagacccagccgagccagtgcacgcggtgaggcggaccggccggctaggcccaaggttcaactacgagctttttaacctcaacaactttaatatacgctattggagctggaattaccgcggctgctggcaccagacttgccctccaattgttcctcgttaagggatttaaattgtactcattccaattacaagacccgaaagagccctgtatcagtatttattgtcactacctccccgtgtcgggattgggtaatttgcgcgcctgctgccttcctttggatgtagtagccgtttctcaggctccttctccggggtcgagccctaaccctccgttacccgttgtcaccacggctggccaagacccagccgtcgaaagttgatagggcagaaatttgaatgaaccatcgccggcgcaaggccgtgcgattcgagaagttattatgaatcaccagagagccccgaagggcattggtttttaatctaataaatacatcccttccgaagtcgggatttttagcatgtattagctctagaattaccacggttatccatgtagtaaggtactatcaaataaacgataactgatttaatgagccattcgcagtttcgcggtataattgcttatacttagacatgcatggcttaatctttgagacaagcatatgactact

SEQ ID NO: 57 - DNA, 925 bp, Chaetomium globosum
  source 1..925: mol_type = genomic DNA
cttccgtcaatttctttaagtttcagccttgcgaccatactcccccaggagcccaaacattttgatttatcgtaaggtgccgaacgggtcaaaaaataacgccgtccgatccctaatcggcatagtttaggttaagactacgacggtatctgatcgtattcgatcccctaactttcgttcctgattaatgaaaacatccttggcaaatgctttcgcagtagttagtcttcaataaatccaagaatttcacctctgacaattgaatactgatgcccccgactgtccctattaatcattacggcggtcctagaaaccaacaaaatagaaccacacgtcctattctattattccatgctaatgtattcgagcataggccttctttaagcgatctaatttgttcagagtaaaagtcctggttccccggcacacccagtgaagggcatgcggttctccagaaggaaagacccagccgagccagtgcacgcggtgaggcggaccggccggctaggcccaaggttcaactacgagctttttaacctcaacaactttaatatacgctattggagctggaattaccgcggctgctggcaccagacttgccctccaattgttcctcgttaagggatttaaattgtactcattccaattacaagacccgaaagagccctgtatcagtatttattgtcactacctccccgtgtcgggattgggtaatttgcgcgcctgctgccttcctttggatgtagtagccgtttctcaggctccttctccggggtcgagccctaaccctccgttacccgttgtcaccacggctggccaagacccagccgtcgaaagttgatagggcagaaatttgaatgaaccatcgccggcgcaaggccgtgcgattcgagaagttattatgaatcaccagagagccccgaag

SEQ ID NO: 58 - DNA, 518 bp, Chaetomium globosum
  source 1..518: mol_type = genomic DNA
gttcacctccagaccggccagtgcgtaagttggaccgaatcgaacattacgaccgaccggccgcgcaggataactgacatggagctctctagggtaaccaaatcggtgccgctttctggtacgtccaagcaaagcaaacactcttggctgatgacaatcgagactgacttcttttcaggcagaccatctctggcgagcacggcctcgacagcaatggcgtgtatgtgggcatgacagttcccaaccgataaatccccgctcaccgcttcgataggtacaacggcacctccgagctccagctcgagcgtatgaacgtgtacttcaacgaggtcagtcgggtcaaataattttacacgaccgagtgatggcgtgctcatagtattatacaggcttccggcaacaagtatgttcctcgcgctgtcctcgtcgacttggagcccggcaccatggatgccgtccgtgccggccccttcggccagctcttccgcccggacaacttcgtcttcggccagtcgggt

SEQ ID NO: 59 - DNA, 568 bp, Chaetomium globosum
  source 1..568: mol_type = genomic DNA
gaggaggaggaggagaggttggagagggaggcgttgcgtgccgaggcgctttgtgaggtcaggcgggttatggcgctgctggaggatacgctgcttgcggacgggcgggagtgggttttgggcggtggtggtggcggtgatggtggtggcagtgagggtgcgagaaaagggccgacgttggcggatatcgaggccgtgtgggtgcttcactggatgattggcattcctggtgcgctgttcaacgccgggtatgtgagcgccgagcggtttccgcgggtgtatgcgtgggtggcgcggtttcaggcggcggttggggcggcgaaggccggggtggtggtgaagggcatgagcggggaggaggcggcggtagtgttgaaggggcagagagaaggggtaggatattttgagaaggagggggaggtggacgccgcggacccgatcgtcaaggtgtacggattggagaaagggagcagggtcgaggtgtggccgacggactccggggctgggcatcgggatcagggctgcctggtgagcctcgacgccgaggaaatagtctgggagacggacg

SEQ ID NO: 60 - DNA, 1503 bp, Exserohilum rostrata
  source 1..1503: mol_type = genomic DNA
tcttggtcatttagaggaagtaaaagtcgtaacaaggtctccgtaggtgaacctgcggagggatcattacacaacaaaaatatgagggtgtggtttgctggcaacagcgtccgccccaagtatttttcacccatgtcttttgcgcactttttgtttcctgggcgagttcgctcgccaccaggacccaaccataaacctttttttatgcagttgcaatcagcgtcagtataataattcaatttattaaaactttcaacaacggatctcttggttctggcatcgatgaagaacgcagcgaaatgcgatacgtagtgtgaattgcagaattcagtgaatcatcgaatctttgaacgcacattgcgccctttggtattccaaagggcatgcctgttcgagcgtcatttgtaccctcaagctttgcttggtgttgggcgtctttttgtctctccccttgttgggggagactcgccttaaaacgattggcagccgacctactggttttcggagcgcagcacaaatttgcgccttccaatccacggggcggcatccagcaagcctttgttttctataacaaatccacattttgacctcggatcaggtagggatacccgctgaacttaagcatatcaataagcggaggaaaagaaaccaacagggattgccctagtaacggcgagtgaagcggcaacagctcaaatttgaaatctggctctttcagagtccgagttgtaatttgcagagggcgctttggctttggcagcggtccaagttccttggaacaggacgtcacagagggtgagaatcccgtacgtggtcgctagctattgccgtgtaaagccccttcgacgagtcgagttgtttgggaatgcagctctaaatgggaggtaaatttcttctaaagctaaatattggccagagaccgatagcgcacaagtagagtgatcgaaagatgaaaagcactttggaaagagagtcaaacagcacgtgaaattgttgaaagggaagcgcttgcagccagacttgcttgcagttgctcatccgggcttttgcccggtgcactcttctgcaggcaggccagcatcagtttgggcggtgggataaaggtctctgtcatgtacctctcttcggggaggccttataggggaggcgacataccaccagcctagactgaggtccgcgcatctgctaggatgctggcgtaatggctgtaagcggcccgtcttgaaacacggaccaaggagtctaacatctatgcgagtgtttgggtgtcaagcccgagcgcgtaatgaaagtgaacggaggtgggaacccgcaagggtgcaccatcgaccgatcctgaagtttacggaaggatttgagtaagagcatggctgttgggacccgaaagatggtgaactatgcttgaatagggtgaagccagaggaaactctggtggaggctcgcagcggttctgacgtgcaaatcgatcgtcaaatttgggcataggggcgaaagactaatcga

SEQ ID NO: 61 - DNA, 1197 bp, Exserohilum rostrata
  source 1..1197: mol_type = genomic DNA
cccatggcttgcttgcccatagcagattggtaggtgttacgaggcgactggttgtgatctgggaaaggaatgatactggcgcaaatacccagaatcatggccggatggatttcacagtgagtgtaggcatggatacgaggatctggtaggggcttgagacggcgaagacggtccttaccctctgtggagcgctccgctgcaggtaggcccatcttcatctctcgccattcttctaagtcctcgggagagaatgtaatcatggcagtctcttcctcctcagcatcgaggtattcgacaacaccatcttggataagacctctccagccataagtagcctgctcaacctcctcctgactccatccttgccttgtgctagtctcttgttgttcagccttgagcttgttactaatctccttggtgaagatgaggtggtttcggtttggctttcgaatatcgttctctacaacaaatagaggtctcatgacacgaccagcatctgtgaagatcttgaactctcggtcacgaatgtcacgaatcaaactcatctcgtaagatagagttccgtttcgtcgaagctcctgcacgaccgtaacaagttgttgagcattggaatgaaccccaacccaaacaccattaacgaaaaccttggtcgcatcggggttttggttctggtcgtattcctcgagcagctgcatgttacgttgcgtcatgaagtcgataatgggcgacgcatcgctaccgacactgacgtaacacatgagagacaagttcttgaccagaccgcaagcctgtccttcaggcgtctcagcagggcagacaagaccccagtgggagttgtgcagttgacggggcttggccaatttaccatcacgtccaacaggagtatttgttcgacgaagatgggacaatgtggaggcgtaagtgtatcggttcaacacctgcgagacaccagccttggcagatgctgccttcttctggtcaccccagttgcctgtagccagagagtacttcaatccgttcgtgatgatgctggcttttacagccatctgaacgttaaagtcctggttgttctcaacgcaccgctggaggtacttgtagacgtccttggtaagcttcaagaagaggatacggaacaagttggcgattaaaggtccagcaagatccaggcgcttctttccgaaatgatcacggtcatcc

SEQ ID NO: 62 - DNA, 307 bp, Exserohilum rostrata
  source 1..307: mol_type = genomic DNA
cttccaggcatagtaatgtggatattaggtgagagcgaaatataagtgtccctagaagtgatagtgagaaggctatggtgaggttgaagaaggtagatggcatattggtaattatgaacatcatcataatctaatgagtcgaaatcattaatttttttttaaactaattaccatttactctgttcattctaatcctttttgtgttcattcatatgctaggcctagagatagaattgtgactagaataaaggctataattattatagtagaggttttaattgtttgaattgctcatggtagtggaagt

SEQ ID NO: 63 - DNA, 1439 bp, Epicoccum nigrum
  source 1..1439: mol_type = genomic DNA
tcttggtcatttagaggaagtaaaagtcgtaacaaggtttccgtaggtgaacctgcggaaggatcattacctagagtttgtggacttcggtctgctacctcttacccatgtcttttgagtaccttcgtttcctcggcgggtccgcccgccggttggacaacattcaaaccctttgcagttgcaatcagcgtctgaaaaaacttaatagttacaactttcaacaacggatctcttggttctggcatcgatgaagaacgcagcgaaatgcgataagtagtgtgaattgcagaattcagtgaatcatcgaatctttgaacgcacattgcgccccttggtattccatggggcatgcctgttcgagcgtcatttgtaccttcaagctctgcttggtgttgggtgttttgtctcgcctccgcgcgcagactcgccttaaaacaattggcagccggcgtattgatttcggagcgcagtacatctcgcgctttgcactcataacgacgacgtccaaaagtacatttttacactcttgacctcggatcaggtagggatacccgctgaacttaagcatatcaataagcggaggaaaagaaaccaacagggattgccctagtaacggcgagtgaagcggcaacagctcaaatttgaaatctggcgtctttggcgtccgagttgtaatttgcagagggcgctttggcattggcagcggtccaagttccttggaacaggacgtcacagagggtgagaatcccgtacgtggtcgctagcctttaccgtgtaaagccccttcgacgagtcgagttgtttgggaatgcagctctaaatgggaggtaaatttcttctaaagctaaatactggccagagaccgatagcgcacaagtagagtgatcgaaagatgaaaagcactttggaaagagagttaaaaagcacgtgaaattgttgaaagggaagcgcttgcagccagacttgcctgtagttgctcatccgggtttctacccggtgcactcttctacgggcaggccagcatcagtttgggcggttggataaaggtctctgtcatgtacctcccttcggggagatcttataggggagacgacatgcaaccagcctggactgaggtccgcgcatctgctaggatgctggcgtaatggctgtaagcggcccgtcttgaaacacggaccaaggagtctaacatctatgcgagtgtttgggtgtcaagcccgagcgcgtaatgaaagtgaacggaggtgggaacctttcggggtgcaccatcgaccgatcctgatgtcttcggatggatttgagtaagagcatagctgttgggacccgaaagatggtgaactatgcttgaatagggtgaagccagaggaaactctggtggaggctcgcagcggttctgacgtgcaaatcgatcgtcaaatttgggcataggggcgaaagac

SEQ ID NO: 64 - DNA, 383 bp, Epicoccum nigrum
  source 1..383: mol_type = genomic DNA
ccagactggccgaagacgaagttatcgggacggaagagctggccgaaggggccggcgcggacagcgtccattgtaccgggctccaagtcgacgaggacggcacggggaacgaacttgttgccagaggcctgcgggaggtcagcactcgcagtccgtctcaggaaagcgtgtcgtttctagtacctcgttgaagtagacgttcatgcgctcgagctggaggtccgaggtgccgttgtagacaccggagccgtcgaggccatgctcgccggagatggtctgccagaaggcagcaccgatttggttaccctgtcccttgtgagctgccgtccatgagagaacatgcaagtggtgtacttacgcactgaccggtctggaggtgaacc

SEQ ID NO: 65 - DNA, 1496 bp, Curvularia protuberata
  source 1..1496: mol_type = genomic DNA
tcttggtcatttagaggaagtaaaagtcgtaacaaggtctccgtaggtgaacctgcggagggatcattacacaataacatatgaaggctgtacgccgctgcgcccccgggccagttggctgaggctggattatttattacccttgtcttttgcgcacttgttgtttcctgggcgggttcgcccgcctccaggaccacaccataaaccttttttatgcagttgcaatcagcgtcagtacaacaaatgtaaatcatttacaactttcaacaacggatctcttggttctggcatcgatgaagaacgcagcgaaatgcgatacgtagtgtgaattgcagaattcagtgaatcatcgaatctttgaacgcacattgcgccctttggtattccaaagggcatgcctgttcgagcgtcatttgtaccctcaagctttgcttggtgttgggcgtttttgtctttggtttgccaaagactcgccttaaaacgattggcagccggcctcctggttacgcagcgcagcacatttttgcgcttgcaatcagcaagagggcggcactccatcaagactccttctcacgtttgacctcggatcaggtagggatacccgctgaacttaagcatatcaataagcggaggaaaagaaaccaacagggattgccctagtaacggcgagtgaagcggcaacagctcaaatttgaaatctggctcttttagggtccgagttgtaatttgcagagggcgctttggctttggcagcggtccaagttccttggaacaggacgtcacagagggtgagaatcccgtacgtggtcgctagctattgccgtgtaaagccccttcgacgagtcgagttgtttgggaatgcagctctaaatgggaggtaaatttcttctaaagctaaatattggccagagaccgatagcgcacaagtagagtgatcgaaagatgaaaagcactttggaaagagagtcaaacagcacgtgaaattgttgaaagggaagcgcttgcagccagacttgcttgcagttgctcatccgggcttttgcccggtgcactcttctgtaggcaggccagcatcagtttgggcggtgggataaaggtctctgacacgttccttccttcgggttggccatataggggagacgtcataccaccagcctggactgaggtccgcgcatctgctaggatgctggcgtaatggctgtaagcggcccgtcttgaaacacggaccaaggagtctaacatctatgcgagtgtttgggtgtcaagcccgagcgcgtaatgaaagtgaacggaggtgggaacccgcaagggcgcaccatcgaccgatcctgaagtttacggaaggatttgagtaagagcatggctgttgggacccgaaagatggtgaactatgcttgaatagggtgaagccagaggaaactctggtggaggctcgcagcggttctgacgtgcaaatcgatcgtcaaatttgggcataggggcgaaagactaatcga

SEQ ID NO: 66 - DNA, 1010 bp, Curvularia protuberata
  source 1..1010: mol_type = genomic DNA
acaccggcagggccgttccagaggatggtctgcgcctcatcgatggcctccttgtaaagcttgatcgacttctctccacagtcgagacccatccagccatctgggataccatccttgtcctcggcataaccgacgttggcgtccttgtcgaacttgtcggcggtgatgtagtcaacaggcagcacaatcttgacattgttcttcttcgccttctccacgaggtccttgacggtcttgctaccagcctcatcgaacaagctttcaccaatcttgacgccctcgagagtcttcttgaaggtgaaggacatgcctccgcaaatgatcaggctgttgaccttgccaagcaggttgtcgatcaattgaatcttgtcagagaccttggcaccaccaaggatggcgaggaaaggtcgcttggggttctcaagcgcttgtgcaaagtaatcaagctccttcttgacaaggaagccagaggccttttgtgggaggtcgacaccgaccatggagctgtgcgcgcggtgagcagtaccaaaagcgtcgtctgtaaaccgtcagcctcgtgctttcgcccatgaattcatagttacttactaatgtagacgtcgcccagagcagtcagtcccttcctaaactcatcgaccttgctcttgtcgaccttctgcttcttgcccgcatcatccttgtagctaccctcctcctcagcgtggaagcgcaggttctcgaggaggatgacctgaccaccgctagcgttgttgacggtatcctctaccgacttgccgacgcagtcgtcggtgaaggtaacgctcttgccgaggagcttctcgagttcgggaacaaccggcttgaggctgtacttcgcattgggcttaccgtctggccggccaaggtgggacatgagaatgacggccttggcgccattgtcgacggcgtacttgattgtgggaagtgcgccaacaatgcgctggttgttggtgatcttcttgtcggcgtcgagagggacgttgaagtcgacc

SEQ ID NO: 67 - DNA, 1443 bp, Cladosporium cladosporioides
  source 1..1443: mol_type = genomic DNA
tcttggtcatttagaggaagtaaaagtcgtaacaaggtctccgtaggtgaacctgcggagggatcattacaagtgaccccggtctaaccaccgggatgttcataaccctttgttgtccgactctgttgcctccggggcgaccctgccttcgggcgggggctccgggtggacacttcaaactcttgcgtaactttgcagtctgagtaaacttaattaataaattaaaacttttaacaacggatctcttggttctggcatcgatgaagaacgcagcgaaatgcgataagtaatgtgaattgcagaattcagtgaatcatcgaatctttgaacgcacattgcgccccctggtattccggggggcatgcctgttcgagcgtcatttcaccactcaagcctcgcttggtattgggcatcgcggtccgccgcgtgcctcaaatcgaccggctgggtcttctgtcccctaagcgttgtggaaactattcgctaaagggtgttcgggaggctacgccgtaaaacaaccccatttctaaggttgacctcggatcaggtagggatacccgctgaacttaagcatatcaataagcggaggaaaagaaaccaacagggattgctctagtaacggcgagtgaagcagcaatagctcaaatttgaaatctggcgtcttcgacgtccgagttgtaatttgtagaggatgcttctgagtaaccaccgacctaagttccttggaacaggacgtcatagagggtgagaatcccgtatgcggtcggaaaggtgctctatacgtagctccttcgacgagtcgagttgtttgggaatgcagctctaaatgggaggtaaatttcttctaaagctaaatattggccagagaccgatagcgcacaagtagagtgatcgaaagatgaaaagcactttggaaagagagttaaaaagcacgtgaaattgttaaaagggaagggattgcaaccagacttgctcgcggtgttccgccggtcttctgaccggtctactcgccgcgttgcaggccagcatcgtctggtgccgctggataagacttgaggaatgtagctccttcgggagtgttatagcctcttgtgatgcagcgagcgccgggcgaggtccgcgcttcggctaggatgctggcgtaatggtcgtaatccgcccgtcttgaaacacggaccaaggagtctaacatctatgcgagtgttcgggtgtcaaacccctacgcgtaatgaaagtgaacggaggtgagaaccgcaaggtgcatcatcgaccgatcctgatgtcttcggatggatttgagtaagagcatagctgttgggacccgaaagatggtgaactatgcctgaatagggtgaagccagaggaaactctggtggaggctcgcagcggttctgacgtgcaaatcgatcgtcaaatttgggtataggggcgaaagactaatcg

SEQ ID NO: 68 - DNA, 1435 bp, Cladosporium oxysporum
  source 1..1435: mol_type = genomic DNA
tcttggtcatttagaggaagtaaaagtcgtaacaaggtctccgtaggtgaacctgcggagggatcattacaagtgaccccggtctaaccaccgggatgttcataaccctttgttgtccgactctgttgcctccggggcgaccctgccttcgggcgggggctccgggtggacacttcaaactcttgcgtaactttgcagtctgagtaaacttaattaataaattaaaacttttaacaacggatctcttggttctggcatcgatgaagaacgcagcgaaatgcgataagtaatgtgaattgcagaattcagtgaatcatcgaatctttgaacgcacattgcgccccctggtattccggggggcatgcctgttcgagcgtcatttcaccactcaagcctcgcttggtattgggcaacgcggtccgccgcgtgcctcaaatcgaccggctgggtcttctgtcccctaagcgttgtggaaactattcgctaaagggtgctcgggaggctacgccgtaaaacaaacccatttctaaggttgacctcggatcaggtagggatacccgctgaacttaagcatatcaataagcggaggaaaagaaaccaacagggattgctctagtaacggcgagtgaagcagcaatagctcaaatttgaaatctggcgtcttcgacgtccgagttgtaatttgtagaggatgcttctgagtaaccaccgacctaagttccttggaacaggacgtcatagagggtgagaatcccgtatgcggtcggaaaggtgctctatacgtagctccttcgacgagtcgagttgtttgggaatgcagctctaaatgggaggtaaatttcttctaaagctaaatattggccagagaccgatagcgcacaagtagagtgatcgaaagatgaaaagcactttggaaagagagttaaaaagcacgtgaaattgttaaaagggaagggattgcaaccagacttgctcgcggtgttccgccggtcttctgaccggtctactcgccgcgttgcaggccagcatcgtctggtgccgctggataagacttgaggaatgtagctccctcgggagtgttatagcctcttgtgatgcagcgagcgccgggcgaggtccgcgcttcggctaggatgctggcgtaatggtcgtaatccgcccgtcttgaaacacggaccaaggagtctaacatctatgcgagtgttcgggtgtcaaacccctacgcgtaatgaaagtgaacggaggtgagaaccgcaaggtgcatcatcgaccgatcctgatgtcttcggatggatttgagtaagagcatagctgttgggacccgaaagatggtgaactatgcctgaatagggtgaagccagaggaaactctggtggaggctcgcagcggttctgacgtgcaaatcgatcgtcaaatttgggtataggggcgaaag

SEQ ID NO: 69 - DNA, 1439 bp, Paecilomyces inflatus
  source 1..1439: mol_type = genomic DNA
tcttggtcatttagaggaagtaaaagtcgtaacaaggtctccgttggtgaaccagcggagggatcattacagagtttaacgactcccaaaccactgtgaacatacccgtaccgttgcctcggcgggcggccccagggcggggccgcagcctccccagcggaggcgcccgccgcaggtcgcaaaactataactatatttagtggcatctctgagtaacttccaaacaatcaaaactttcaacaacggatctcttggttctggcatcgatgaagaacgcagcgaaatgcgataagtaatgtgaattgcagaattcagtgaatcatcgaatctttgaacgcacattgcgcccgccagcattctggcgggcatgcctgtccgagcgtcatttcaaccctcaagccctgcttggtgttggggcactacgcgcgagcgtaggccctcaaaatcagtggcggacccgctggaggtccgggcgtagtaacacatctcgcccgaggtccccagcgtgcccctgccgttaaacccccaaatttacagaaggttgacctcggatcaggtaggaatacccgctgaacttaagcatatcaataagcggaggaaaagaaaccaacagggattgccctagtaacggcgagtgaagcggcaacagctcgaatttgaaatctggcctcggcccgagttgtaatctgtagaggatgcttttggcgcggtgccttccgagtgccctggaacgggacgccacagagggtgagagccccgtatggtcggacaccaagcctgtgtaaagctccttcgacgagtcgggtagcttgggaatgctgctctaagtgggaggtaaacttcttctaaagctaaatactggccagagaccgatagcgcacaagtagagtgatcgaaagatgaaaagcactttgaaaagagggtcaaatagtacgtgaaattgttgaaagggaagcgctcatgaccagacttgcgccgggctgatcatccagtggtctccactggtgcactctgcccggctcaggccagcgtcggctgtcacggggggacaaaagcactgggaaagtagctctctccggggagtgttatagccctatgcagaatacccccgcggcggccgaggtccgcgctctgcaaggacgctggcgtaatggtcatcagcgacccgtcttgaaacacggaccaaggagtcgaggttttgcgcgagtgttcgggtgcaaagccccagcgcgtaattaaagtgaacgtaggtgagagcttcggcgcatcatcgaccgatcctgatgtattcggatggatttgagtaggagcgtaaagcctcggacccgaaagatggtgaactatgcctgtatagggtgaagccagaggaaactctggtggaggctcgcagcggttctgacgtgcaaatcgatcgtcaaatatgggcatgggggcgaaag

SEQ ID NO: 70 - DNA, 1443 bp, Epicoccum nigrum
  source 1..1443: mol_type = genomic DNA
tcttggtcatttagaggaagtaaaagtcgtaacaaggtttccgtaggtgaacctgcggaaggatcattacctagagtttgtggacttcggtctgctacctcttacccatgtcttttgagtaccttcgtttcctcggcgggtccgcccgccggttggacaacattcaaaccctttgcagttgcaatcagcgtctgaaaaaacttaatagttacaactttcaacaacggatctcttggttctggcatcgatgaagaacgcagcgaaatgcgataagtagtgtgaattgcagaattcagtgaatcatcgaatctttgaacgcacattgcgccccttggtattccatggggcatgcctgttcgagcgtcatttgtaccttcaagctctgcttggtgttgggtgttttgtctcgcctccgcgcgcagactcgccttaaaacaattggcagccggcgtattgatttcggagcgcagtacatctcgcgctttgcactcataacgacgacgtccaaaagtacatttttacactcttgacctcggatcaggtagggatacccgctgaacttaagcatatcaataagcggaggaaaagaaaccaacagggattgccctagtaacggcgagtgaagcggcaacagctcaaatttgaaatctggcgtctttggcgtccgagttgtaatttgcagagggcgctttggcattggcagcggtccaagttccttggaacaggacgtcacagagggtgagaatcccgtacgtggtcgctagcctttaccgtgtaaagccccttcgacgagtcgagttgtttgggaatgcagctctaaatgggaggtaaatttcttctaaagctaaatactggccagagaccgatagcgcacaagtagagtgatcgaaagatgaaaagcactttggaaagagagttaaaaagcacgtgaaattgttgaaagggaagcgcttgcagccagacttgcctgtagttgctcatccgggtttctacccggtgcactcttctacgggcaggccagcatcagtttgggcggttggataaaggtctctgtcatgtacctcccttcggggagatcttataggggagacgacatgcaaccagcctggactgaggtccgcgcatctgctaggatgctggcgtaatggctgtaagcggcccgtcttgaaacacggaccaaggagtctaacatctatgcgagtgtttgggtgtcaagcccgagcgcgtaatgaaagtgaacggaggtgggaacctttcggggtgcaccatcgaccgatcctgatgtcttcggatggatttgagtaagagcatagctgttgggacccgaaagatggtgaactatgcttgaatagggtgaagccagaggaaactctggtggaggctcgcagcggttctgacgtgcaaatcgatcgtcaaatttgggcataggggcgaaagactaat

SEQ ID NO: 71 - DNA, 608 bp, Epicoccum nigrum
  misc_feature 113..126: note = n is a, c, g, or t
  source 1..608: mol_type = genomic DNA
ctcctcctcctcctcctgatcgaactcgccccccaccaactccaccagcccacccagccgcccaaaaacctccccatccccgctagccgcccccatggcccggacaagcagcnnnnnnnnnnnnnngtccgggatggccttaggttcgctctcgagctgctccagccgcgacaggacatgcagcagctccctgcgcagcgagtccggcgccggcatgcggccccgcagcggctggtcggcgatgtatgtcttgagcgggagcgcggcgcgcaggatgaggtagggcgccgctgcctgggcgagtttgatgtgcgagtgcgagggcgagggcgaggtactggcggggcgtgcggccacgagggcgaagagggaggccgtgcaggtgtagctcatctttgtgcgcaaggtggcggggaggacggccgtctggccggtgcggacggagaggaggttggcgaggggcgaggtggtgatgggagggagttctccttgtacgggagtgtggatgagggaggtggtgaagaggttgcgggcgtatgtcctgcggagggtgtcggggagggagggggagtttagagggccgctgatcaagtcgcgtagctctgtga